European Patent Application EP 4 170 022 A1, published April 26, 2023. Title: RECOMBINANT AFRICAN SWINE FEVER VIRUS AND USES THEREOF. Applicant: CONSEJO SUPERIOR DE INVESTIGACIONES CIENTÍFICAS /  Icahn School of Medicine at Mount Sinai. The sequence listing filed with the application follows.

SEQUENCE LISTING (44 sequences)

SEQ ID NO: 1 - DNA, 23 bp, Artificial Sequence
  miRNA target sequence
tccataaagtaggaaacactaca

SEQ ID NO: 2 - RNA, 23 nt, Artificial Sequence
  miRNA target sequence
uccauaaaguaggaaacacuaca

SEQ ID NO: 3 - RNA, 22 nt, Sus scrofa
uguaguguuuccuacuuuaugg

SEQ ID NO: 4 - DNA, 112 bp, Artificial Sequence
  miRNA target sequence x4
gtcgactccataaagtaggaaacactacacgattccataaagtaggaaacactacaaccggttccataaagtaggaaacactacatcactccataaagtaggaaacactaca

SEQ ID NO: 5 - DNA, 23 bp, Artificial Sequence
  gRNA_CP123L-0
ataaccagtgtcccagtcgaggg

SEQ ID NO: 6 - DNA, 23 bp, Artificial Sequence
  gRNA_CP123L-1
gcttttttggcgaatcataaggg

SEQ ID NO: 7 - DNA, 19 bp, Artificial Sequence
  oligo
gagacccaagctggctagc

SEQ ID NO: 8 - DNA, 19 bp, Artificial Sequence
  oligo
aacgcgtatatctggcccg

SEQ ID NO: 9 - DNA, 57 bp, Artificial Sequence
  Oligo
ccagatatacgcgttgacattgattattgactagttattaatagtaatcaattacgg

SEQ ID NO: 10 - DNA, 38 bp, Artificial Sequence
  oligo
gccagcttgggtctcttacttgtacagctcgtccatgc

SEQ ID NO: 11 - DNA, 49 bp, Artificial Sequence
  oligo
tatttaataaaaacaataaattatttttataacattatataggtcgcca

SEQ ID NO: 12 - DNA, 19 bp, Artificial Sequence
  oligo
aacgcgtatatctggcccg

SEQ ID NO: 13 - DNA, 46 bp, Artificial Sequence
  oligo
ccagatatacgcgttgtcgactccataaagtaggaaacactacacg

SEQ ID NO: 14 - DNA, 44 bp, Artificial Sequence
  oligo
tgtttttattaaatataagatacattgatgagtttggacaaacc

SEQ ID NO: 15 - DNA, 21 bp, Artificial Sequence
  oligo
cttctgaggcggaaagaacca

SEQ ID NO: 16 - DNA, 19 bp, Artificial Sequence
  oligo
aacgcgtatatctggcccg

SEQ ID NO: 17 - DNA, 47 bp, Artificial Sequence
  oligo
ccagatatacgcgttaaaccattctatgaaaaaaatggttgaacagc

SEQ ID NO: 18 - DNA, 50 bp, Artificial Sequence
  oligo
tttccgcctcagaagtcatatacagaaaatagtgtgctgacctatatcac

SEQ ID NO: 19 - DNA, 27 bp, Artificial Sequence
  oligo
aattctgtggaatgtgtgtcagttagg

SEQ ID NO: 20 - DNA, 19 bp, Artificial Sequence
  oligo
ggggataccccctagagcc

SEQ ID NO: 21 - DNA, 43 bp, Artificial Sequence
  oligo
ctagggggtatccccaaaaaaacatctgcaagcttttttggat

SEQ ID NO: 22 - DNA, 32 bp, Artificial Sequence
  oligo
acattccacagaattatgccctcgactgggac

SEQ ID NO: 23 - DNA, 50 bp, Artificial Sequence
  oligo
tttgttatataagtaacgtttttttttattttttataattcgaatgaaga

SEQ ID NO: 24 - DNA, 30 bp, Artificial Sequence
  oligo
ttaggaaataaagtcgtagcaagatggttt

SEQ ID NO: 25 - DNA, 46 bp, Artificial Sequence
  oligo
gactttatttcctaagtcgactccataaagtaggaaacactacacg

SEQ ID NO: 26 - DNA, 34 bp, Artificial Sequence
  oligo
tacttatataacaaaatgccctcgactgggacac

SEQ ID NO: 27 - DNA, 29 bp, Artificial Sequence
  oligo
gcagctgattacggaagaaaaaaaaattg

SEQ ID NO: 28 - DNA, 34 bp, Artificial Sequence; identical to SEQ ID NO: 26
  oligo

SEQ ID NO: 29 - DNA, 29 bp, Artificial Sequence
  oligo
gcagctgattacggaagaaaaaaaaattg

SEQ ID NO: 30 - DNA, 20 bp, Artificial Sequence
  oligo
gaacttgtggccgtttacgt

SEQ ID NO: 31 - DNA, 29 bp, Artificial Sequence
  primer
gcagctgattacggaagaaaaaaaaattg

SEQ ID NO: 32 - DNA, 20 bp, Artificial Sequence
  primer
gaacttgtggccgtttacgt

SEQ ID NO: 33 - DNA, 21 bp, Artificial Sequence
  primer
ggcccgaggttatctagagtc

SEQ ID NO: 34 - DNA, 18 bp, Artificial Sequence
  primer
tcaaaaccaacccggtca

SEQ ID NO: 35 - DNA, 26 bp, Artificial Sequence
  primer
aaaaatgataatgaaaccaatgaatg

SEQ ID NO: 36 - DNA, 20 bp, Artificial Sequence
  primer
atgagggctcttgctcaaac

SEQ ID NO: 37 - DNA, 22 bp, Artificial Sequence
  primer
ggtttcatccattcaattaggc

SEQ ID NO: 38 - DNA, 20 bp, Artificial Sequence
  primer
cgctctctgttggccttaaa

SEQ ID NO: 39 - DNA, 20 bp, Artificial Sequence
  primer
tagccgacgtggcctattac

SEQ ID NO: 40 - DNA, 19 bp, Artificial Sequence
  primer
gcaccagaaggtcctgaca

SEQ ID NO: 41 - DNA, 159 bp, Artificial Sequence
  miRNA target
gtggcagtattaaaccatcttgctacgactttatttcctagtcgactccataaagtaggaaacactacacgattccataaagtaggaaacactacaaccggttccataaagtaggaaacactacatcactccataaagtaggaaacactacactcgagg

SEQ ID NO: 42 - DNA, 160 bp, Artificial Sequence
  miRNA target
gtggcagtattaaaccatcttgctacgactttatttcctaagtcgactccataaagtaggaaacactacacgattccataaagtaggaaacactacaaccggttccataaagtaggaaacactacatcactccataaagtaggaaacactacactcgagg

SEQ ID NO: 43 - DNA, 121 bp, Artificial Sequence
  miRNA Target
taagtcgactccataaagtaggaaacactacacgattccataaagtaggaaacactacaaccggttccataaagtaggaaacactacatcactccataaagtaggaaacactacactcgag

SEQ ID NO: 44 - protein, 13 aa, African swine fever virus
CGSIKPSCYDFIS